European Patent Specification EP 3 305 762 B1, published August 5, 2026. Title: Nonpeptide GAPDH aggregation inhibitor. Applicant: Osaka Prefecture University Public Corporation. The sequence listing filed with the application follows.

SEQUENCE LISTING (1 sequence)

SEQ ID NO: 1 - protein, 10 aa, Artificial Sequence
  GAPDH Aggregation inhibitor
SNASCTTNAL